European Patent Specification EP 3 715 346 B1, published January 3, 2024. Title: THIAZOLYL-CONTAINING COMPOUNDS FOR TREATING PROLIFERATIVE DISEASES. Applicant: Dana-Farber Cancer Institute, Inc. The sequence listing filed with the application follows.

SEQUENCE LISTING (235 sequences)

SEQ ID NO: 1 - protein, 18 aa, Artificial Sequence
  Synthetic Polypeptide
LMTGDTYTAHAGAKFPIK

SEQ ID NO: 2 - protein, 22 aa, Artificial Sequence
  Synthetic Polypeptide
YSLTVAVKTLKEDTMEVEEFLK

SEQ ID NO: 3 - protein, 25 aa, Artificial Sequence
  Synthetic Polypeptide
TVSVAVKCLKPDVLSQPEAMDDFIR

SEQ ID NO: 4 - protein, 13 aa, Artificial Sequence
  Synthetic Polypeptide
ATVFLNPAACKGK

SEQ ID NO: 5 - protein, 10 aa, Artificial Sequence
  Synthetic Polypeptide
GTFGKVILVK

SEQ ID NO: 6 - protein, 10 aa, Artificial Sequence
  Synthetic Polypeptide
GTFGKVILVR

SEQ ID NO: 7 - protein, 16 aa, Artificial Sequence
  Synthetic Polypeptide
DLKPENVLLDAHMNAK

SEQ ID NO: 8 - protein, 16 aa, Artificial Sequence
  Synthetic Polypeptide
DLKSNNIFLHEGLTVK

SEQ ID NO: 9 - protein, 28 aa, Artificial Sequence
  Synthetic Polypeptide
QLVKGRDDLRQDAVMQQVFQMCNTLLQR

SEQ ID NO: 10 - protein, 9 aa, Artificial Sequence
  Synthetic Polypeptide
FYIMMCKPK

SEQ ID NO: 11 - protein, 10 aa, Artificial Sequence
  Synthetic Polypeptide
FILALKVLFK

SEQ ID NO: 12 - protein, 16 aa, Artificial Sequence
  Synthetic Polypeptide
DIKPENLLLGSAGELK

SEQ ID NO: 13 - protein, 10 aa, Artificial Sequence
  Synthetic Polypeptide
GKFGNVYLAR

SEQ ID NO: 14 - protein, 12 aa, Artificial Sequence
  Synthetic Polypeptide
SHFIVALKVLFK

SEQ ID NO: 15 - protein, 17 aa, Artificial Sequence
  Synthetic Polypeptide
IIDSEYTAQEGAKFPIK

SEQ ID NO: 16 - protein, 16 aa, Artificial Sequence
  Synthetic Polypeptide
DLKSNNIFLHEDLTVK

SEQ ID NO: 17 - protein, 18 aa, Artificial Sequence
  Synthetic Polypeptide
YVLDDEYTSSVGSKFPVR

SEQ ID NO: 18 - protein, 9 aa, Artificial Sequence
  Synthetic Polypeptide
LFAVKCIPK

SEQ ID NO: 19 - protein, 16 aa, Artificial Sequence
  Synthetic Polypeptide
IPTGQEYAAKIINTKK

SEQ ID NO: 20 - protein, 14 aa, Artificial Sequence
  Synthetic Polypeptide
TSTQEYAAKIINTK

SEQ ID NO: 21 - protein, 19 aa, Artificial Sequence
  Synthetic Polypeptide
DLKPENLLYATPAPDAPLK

SEQ ID NO: 22 - protein, 16 aa, Artificial Sequence
  Synthetic Polypeptide
DIKPSNLLVGEDGHIK

SEQ ID NO: 23 - protein, 15 aa, Artificial Sequence
  Synthetic Polypeptide
ETGQQFAVKIVDVAK

SEQ ID NO: 24 - protein, 16 aa, Artificial Sequence
  Synthetic Polypeptide
DLKPQNLLIDDKGTIK

SEQ ID NO: 25 - protein, 11 aa, Artificial Sequence
  Synthetic Polypeptide
DVKPSNFLYNR

SEQ ID NO: 26 - protein, 16 aa, Artificial Sequence
  Synthetic Polypeptide
DLKPANILVMGEGPER

SEQ ID NO: 27 - protein, 16 aa, Artificial Sequence
  Synthetic Polypeptide
DLKPQNLLINTEGAIK

SEQ ID NO: 28 - protein, 16 aa, Artificial Sequence
  Synthetic Polypeptide
DLKPENILVTSGGTVK

SEQ ID NO: 29 - protein, 11 aa, Artificial Sequence
  Synthetic Polypeptide
DLKPQNLLINR

SEQ ID NO: 30 - protein, 16 aa, Artificial Sequence
  Synthetic Polypeptide
DLKPQNILVTSSGQIK

SEQ ID NO: 31 - protein, 16 aa, Artificial Sequence
  Synthetic Polypeptide
DLKPNNLLLDENGVLK

SEQ ID NO: 32 - protein, 11 aa, Artificial Sequence
  Synthetic Polypeptide
DMKAANVLITR

SEQ ID NO: 33 - protein, 12 aa, Artificial Sequence
  Synthetic Polypeptide
DIKCSNILLNNR

SEQ ID NO: 34 - protein, 12 aa, Artificial Sequence
  Synthetic Polypeptide
DIKPENLLLDER

SEQ ID NO: 35 - protein, 19 aa, Artificial Sequence
  Synthetic Polypeptide
DLKPENVLLSSQEEDCLIK

SEQ ID NO: 36 - protein, 13 aa, Artificial Sequence
  Synthetic Polypeptide
DIKPDNFLMGIGR

SEQ ID NO: 37 - protein, 14 aa, Artificial Sequence
  Synthetic Polypeptide
DVKPDNFLMGLGKK

SEQ ID NO: 38 - protein, 11 aa, Artificial Sequence
  Synthetic Polypeptide
KIGCGNFGELR

SEQ ID NO: 39 - protein, 15 aa, Artificial Sequence
  Synthetic Polypeptide
DVKPENFLVGRPGTK

SEQ ID NO: 40 - protein, 14 aa, Artificial Sequence
  Synthetic Polypeptide
DVKPHNVMIDHQQK

SEQ ID NO: 41 - protein, 25 aa, Artificial Sequence
  Synthetic Polypeptide
LTHTDLKPENILFVQSDYTEAYNPK

SEQ ID NO: 42 - protein, 26 aa, Artificial Sequence
  Synthetic Polypeptide
LTHTDLKPENILFVNSDYELTYNLEK

SEQ ID NO: 43 - protein, 23 aa, Artificial Sequence
  Synthetic Polypeptide
YEIVGNLGEGTFGKVVECLDHAR

SEQ ID NO: 44 - protein, 13 aa, Artificial Sequence
  Synthetic Polypeptide
GAFGKVYLAQDIK

SEQ ID NO: 45 - protein, 16 aa, Artificial Sequence
  Synthetic Polypeptide
DIKCSNILLNNSGQIK

SEQ ID NO: 46 - protein, 22 aa, Artificial Sequence
  Synthetic Polypeptide
VSDFGLTKEASSTQDTGKLPVK

SEQ ID NO: 47 - protein, 21 aa, Artificial Sequence
  Synthetic Polypeptide
IDPVPNTHPLLVFVNPKSGGK

SEQ ID NO: 48 - protein, 25 aa, Artificial Sequence
  Synthetic Polypeptide
ATFSFCVSPLLVFVNSKSGDNQGVK

SEQ ID NO: 49 - protein, 16 aa, Artificial Sequence
  Synthetic Polypeptide
DLKSPNMLITYDDVVK

SEQ ID NO: 50 - protein, 14 aa, Artificial Sequence
  Synthetic Polypeptide
KGGSWIQEINVAEK

SEQ ID NO: 51 - protein, 13 aa, Artificial Sequence
  Synthetic Polypeptide
EHPFLVKGGEDLR

SEQ ID NO: 52 - protein, 12 aa, Artificial Sequence
  Synthetic Polypeptide
YIKYNSNSGFVR

SEQ ID NO: 53 - protein, 9 aa, Artificial Sequence
  Synthetic Polypeptide
IPVAIKELR

SEQ ID NO: 54 - protein, 22 aa, Artificial Sequence
  Synthetic Polypeptide
YLQDDTSDPTYTSSLGGKIPVR

SEQ ID NO: 55 - protein, 22 aa, Artificial Sequence
  Synthetic Polypeptide
FLEDDTSDPTYTSALGGKIPIR

SEQ ID NO: 56 - protein, 16 aa, Artificial Sequence
  Synthetic Polypeptide
DLKPSNLLINTTCDLK

SEQ ID NO: 57 - protein, 16 aa, Artificial Sequence
  Synthetic Polypeptide
DLKPSNLLLNTTCDLK

SEQ ID NO: 58 - protein, 17 aa, Artificial Sequence
  Synthetic Polypeptide
DLKPANLFINTEDLVLK

SEQ ID NO: 59 - protein, 16 aa, Artificial Sequence
  Synthetic Polypeptide
DLKPSNLLVNENCELK

SEQ ID NO: 60 - protein, 17 aa, Artificial Sequence
  Synthetic Polypeptide
TSVAVKTCKEDLPQELK

SEQ ID NO: 61 - protein, 14 aa, Artificial Sequence
  Synthetic Polypeptide
LRADNTLVAVKSCR

SEQ ID NO: 62 - protein, 18 aa, Artificial Sequence
  Synthetic Polypeptide
LIKDDEYNPCQGSKFPIK

SEQ ID NO: 63 - protein, 18 aa, Artificial Sequence
  Synthetic Polypeptide
IQSIAPSLQVITSKQRPR

SEQ ID NO: 64 - protein, 8 aa, Artificial Sequence
  Synthetic Polypeptide
HEIKLPVK

SEQ ID NO: 65 - protein, 24 aa, Artificial Sequence
  Synthetic Polypeptide
VAIKTLKPGTMSPESFLEEAQIMK

SEQ ID NO: 66 - protein, 19 aa, Artificial Sequence
  Synthetic Polypeptide
QGAKFPIKWTAPEAALYGR

SEQ ID NO: 67 - protein, 16 aa, Artificial Sequence
  Synthetic Polypeptide
DLKVENLLLSNQGTIK

SEQ ID NO: 68 - protein, 16 aa, Artificial Sequence
  Synthetic Polypeptide
DIKGANLLLTLQGDVK

SEQ ID NO: 69 - protein, 16 aa, Artificial Sequence
  Synthetic Polypeptide
DLKPVNIFLDSDDHVK

SEQ ID NO: 70 - protein, 17 aa, Artificial Sequence
  Synthetic Polypeptide
DIKPQNLLVDPDTAVLK

SEQ ID NO: 71 - protein, 17 aa, Artificial Sequence
  Synthetic Polypeptide
DIKPQNLLLDPDTAVLK

SEQ ID NO: 72 - protein, 16 aa, Artificial Sequence
  Synthetic Polypeptide
DIKGANILINDAGEVR

SEQ ID NO: 73 - protein, 15 aa, Artificial Sequence
  Synthetic Polypeptide
DLKPENIVLQDVGGK

SEQ ID NO: 74 - protein, 15 aa, Artificial Sequence
  Synthetic Polypeptide
DLKPENIVLQQGEQR

SEQ ID NO: 75 - protein, 19 aa, Artificial Sequence
  Synthetic Polypeptide
SGELVAVKVFNTTSYLRPR

SEQ ID NO: 76 - protein, 12 aa, Artificial Sequence
  Synthetic Polypeptide
WQGNDIVVKVLK

SEQ ID NO: 77 - protein, 15 aa, Artificial Sequence
  Synthetic Polypeptide
ISMADVKFSFQCPGR

SEQ ID NO: 78 - protein, 27 aa, Artificial Sequence
  Synthetic Polypeptide
AIQFLHQDSPSLIHGDIKSSNVLLDER

SEQ ID NO: 79 - protein, 14 aa, Artificial Sequence
  Synthetic Polypeptide
VEIQNLTYAVKLFK

SEQ ID NO: 80 - protein, 16 aa, Artificial Sequence
  Synthetic Polypeptide
DIKSANILLDEAFTAK

SEQ ID NO: 81 - protein, 17 aa, Artificial Sequence
  Synthetic Polypeptide
DLKPHNILISMPNAHGK

SEQ ID NO: 82 - protein, 38 aa, Artificial Sequence
  Synthetic Polypeptide
ESIFFNSHNVSKPESSSVLTELDKIEGVFERPSDEVIR

SEQ ID NO: 83 - protein, 28 aa, Artificial Sequence
  Synthetic Polypeptide
QLASALSYLEDKDLVHGNVCTKNLLLAR

SEQ ID NO: 84 - protein, 20 aa, Artificial Sequence
  Synthetic Polypeptide
IGDFGLTKAIETDKEYYTVK

SEQ ID NO: 85 - protein, 31 aa, Artificial Sequence
  Synthetic Polypeptide
YDPEGDNTGEQVAVKSLKPESGGNHIADLKK

SEQ ID NO: 86 - protein, 20 aa, Artificial Sequence
  Synthetic Polypeptide
IADFGLAKLLPLDKDYYVVR

SEQ ID NO: 87 - protein, 10 aa, Artificial Sequence
  Synthetic Polypeptide
DLKPSNIVVK

SEQ ID NO: 88 - protein, 14 aa, Artificial Sequence
  Synthetic Polypeptide
NVHTGELAAVKIIK

SEQ ID NO: 89 - protein, 14 aa, Artificial Sequence
  Synthetic Polypeptide
NVNTGELAAIKVIK

SEQ ID NO: 90 - protein, 26 aa, Artificial Sequence
  Synthetic Polypeptide
SKNVFYDNGKVVITDFGLFGISGVVR

SEQ ID NO: 91 - protein, 10 aa, Artificial Sequence
  Synthetic Polypeptide
SKNVFYDNGK

SEQ ID NO: 92 - protein, 9 aa, Artificial Sequence
  Synthetic Polypeptide
ALYATKTLR

SEQ ID NO: 93 - protein, 16 aa, Artificial Sequence
  Synthetic Polypeptide
DIKPDNILIDLDGHIK

SEQ ID NO: 94 - protein, 23 aa, Artificial Sequence
  Synthetic Polypeptide
EGAKFPIKWTAPEAINYGTFTIK

SEQ ID NO: 95 - protein, 16 aa, Artificial Sequence
  Synthetic Polypeptide
DIKPGNLLLTTGGTLK

SEQ ID NO: 96 - protein, 16 aa, Artificial Sequence
  Synthetic Polypeptide
DLKAGNVLMTLEGDIR

SEQ ID NO: 97 - protein, 21 aa, Artificial Sequence
  Synthetic Polypeptide
DLKPHNVLLFTLYPNAAIIAK

SEQ ID NO: 98 - protein, 24 aa, Artificial Sequence
  Synthetic Polypeptide
VAVKTLKPGTMSVQAFLEEANLMK

SEQ ID NO: 99 - protein, 16 aa, Artificial Sequence
  Synthetic Polypeptide
IMHRDVKPSNILVNSR

SEQ ID NO: 100 - protein, 12 aa, Artificial Sequence
  Synthetic Polypeptide
KLIHLEIKPAIR

SEQ ID NO: 101 - protein, 12 aa, Artificial Sequence
  Synthetic Polypeptide
DVKPSNILVNSR

SEQ ID NO: 102 - protein, 18 aa, Artificial Sequence
  Synthetic Polypeptide
HQIMHRDVKPSNILVNSR

SEQ ID NO: 103 - protein, 11 aa, Artificial Sequence
  Synthetic Polypeptide
DVKPSNVLINK

SEQ ID NO: 104 - protein, 11 aa, Artificial Sequence
  Synthetic Polypeptide
DIKPSNILLDR

SEQ ID NO: 105 - protein, 12 aa, Artificial Sequence
  Synthetic Polypeptide
DVKPSNMLVNTR

SEQ ID NO: 106 - protein, 16 aa, Artificial Sequence
  Synthetic Polypeptide
DVKPSNVLINALGQVK

SEQ ID NO: 107 - protein, 12 aa, Artificial Sequence
  Synthetic Polypeptide
DVKPSNILLDER

SEQ ID NO: 108 - protein, 15 aa, Artificial Sequence
  Synthetic Polypeptide
DVKGANLLIDSTGQR

SEQ ID NO: 109 - protein, 31 aa, Artificial Sequence
  Synthetic Polypeptide
ELAVKQVQFDPDSPETSKEVNALECEIQLLK

SEQ ID NO: 110 - protein, 9 aa, Artificial Sequence
  Synthetic Polypeptide
DIKGANILR

SEQ ID NO: 111 - protein, 31 aa, Artificial Sequence
  Synthetic Polypeptide
ELASKQVQFDPDSPETSKEVSALECEIQLLK

SEQ ID NO: 112 - protein, 16 aa, Artificial Sequence
  Synthetic Polypeptide
DIKGANIFLTSSGLIK

SEQ ID NO: 113 - protein, 17 aa, Artificial Sequence
  Synthetic Polypeptide
DIKGDNVLINTYSGVLK

SEQ ID NO: 114 - protein, 17 aa, Artificial Sequence
  Synthetic Polypeptide
DIKGDNVLINTFSGLLK

SEQ ID NO: 115 - protein, 16 aa, Artificial Sequence
  Synthetic Polypeptide
DLKAENLLLDADMNIK

SEQ ID NO: 116 - protein, 19 aa, Artificial Sequence
  Synthetic Polypeptide
EVAIKIIDKTQLNPTSLQK

SEQ ID NO: 117 - protein, 9 aa, Artificial Sequence
  Synthetic Polypeptide
EVAIKIIDK

SEQ ID NO: 118 - protein, 16 aa, Artificial Sequence
  Synthetic Polypeptide
DLKAENLLLDAEANIK

SEQ ID NO: 119 - protein, 16 aa, Artificial Sequence
  Synthetic Polypeptide
DLKPDNLLITSMGHIK

SEQ ID NO: 120 - protein, 16 aa, Artificial Sequence
  Synthetic Polypeptide
DLKPDNLLITSLGHIK

SEQ ID NO: 121 - protein, 11 aa, Artificial Sequence
  Synthetic Polypeptide
GAFGKVYLGQK

SEQ ID NO: 122 - protein, 8 aa, Artificial Sequence
  Synthetic Polypeptide
LYAVKVVK

SEQ ID NO: 123 - protein, 14 aa, Artificial Sequence
  Synthetic Polypeptide
DLKPENLLFDEYHK

SEQ ID NO: 124 - protein, 20 aa, Artificial Sequence
  Synthetic Polypeptide
NCMLRDDMTVCVADFGLSKK

SEQ ID NO: 125 - protein, 9 aa, Artificial Sequence
  Synthetic Polypeptide
KIYSGDYYR

SEQ ID NO: 126 - protein, 13 aa, Artificial Sequence
  Synthetic Polypeptide
DMYDKEYYSVHNK

SEQ ID NO: 127 - protein, 12 aa, Artificial Sequence
  Synthetic Polypeptide
DLKSSNILILQK

SEQ ID NO: 128 - protein, 21 aa, Artificial Sequence
  Synthetic Polypeptide
DLKSNNILLLQPIESDDMEHK

SEQ ID NO: 129 - protein, 12 aa, Artificial Sequence
  Synthetic Polypeptide
DLKSSNILLLEK

SEQ ID NO: 130 - protein, 9 aa, Artificial Sequence
  Synthetic Polypeptide
APVAIKVFK

SEQ ID NO: 131 - protein, 34 aa, Artificial Sequence
  Synthetic Polypeptide
DLKPTNILLGDEGQPVLMDLGSMNQACIHVEGSR

SEQ ID NO: 132 - protein, 24 aa, Artificial Sequence
  Synthetic Polypeptide
DIKLENILLDSNGHVVLTDFGLSK

SEQ ID NO: 133 - protein, 24 aa, Artificial Sequence
  Synthetic Polypeptide
DLKLENVLLDSEGHIVLTDFGLSK

SEQ ID NO: 134 - protein, 22 aa, Artificial Sequence
  Synthetic Polypeptide
ETGQIVAIKQVPVESDLQEIIK

SEQ ID NO: 135 - protein, 22 aa, Artificial Sequence
  Synthetic Polypeptide
ESGQVVAIKQVPVESDLQEIIK

SEQ ID NO: 136 - protein, 16 aa, Artificial Sequence
  Synthetic Polypeptide
DIKAANVLLSEHGEVK

SEQ ID NO: 137 - protein, 39 aa, Artificial Sequence
  Synthetic Polypeptide
TQQVVAIKIIDLEEAEDEIEDIQQEITVLSQCDSSYVTK

SEQ ID NO: 138 - protein, 16 aa, Artificial Sequence
  Synthetic Polypeptide
DIKAANVLLSEQGDVK

SEQ ID NO: 139 - protein, 12 aa, Artificial Sequence
  Synthetic Polypeptide
DIKPDNLLLDSK

SEQ ID NO: 140 - protein, 12 aa, Artificial Sequence
  Synthetic Polypeptide
DIKPDNLLLDAK

SEQ ID NO: 141 - protein, 11 aa, Artificial Sequence
  Synthetic Polypeptide
DIKSQNIFLTK

SEQ ID NO: 142 - protein, 12 aa, Artificial Sequence
  Synthetic Polypeptide
DLKPANVFLDGK

SEQ ID NO: 143 - protein, 11 aa, Artificial Sequence
  Synthetic Polypeptide
SKNIFLTQNGK

SEQ ID NO: 144 - protein, 11 aa, Artificial Sequence
  Synthetic Polypeptide
DLKTQNVFLTR

SEQ ID NO: 145 - protein, 16 aa, Artificial Sequence
  Synthetic Polypeptide
DIKPANVFITATGVVK

SEQ ID NO: 146 - protein, 14 aa, Artificial Sequence
  Synthetic Polypeptide
AACLLDGVPVALKK

SEQ ID NO: 147 - protein, 11 aa, Artificial Sequence
  Synthetic Polypeptide
DLKTQNILLDK

SEQ ID NO: 148 - protein, 11 aa, Artificial Sequence
  Synthetic Polypeptide
DIKTLNIFLTK

SEQ ID NO: 149 - protein, 16 aa, Artificial Sequence
  Synthetic Polypeptide
DIKPGNLLVNSNCVLK

SEQ ID NO: 150 - protein, 34 aa, Artificial Sequence
  Synthetic Polypeptide
DVKAGNILLGEDGSVQIADFGVSAFLATGGDITR

SEQ ID NO: 151 - protein, 16 aa, Artificial Sequence
  Synthetic Polypeptide
DLKPSNLAVNEDCELK

SEQ ID NO: 152 - protein, 13 aa, Artificial Sequence
  Synthetic Polypeptide
QELNKTIWEVPER

SEQ ID NO: 153 - protein, 16 aa, Artificial Sequence
  Synthetic Polypeptide
DLKPGNLAVNEDCELK

SEQ ID NO: 154 - protein, 16 aa, Artificial Sequence
  Synthetic Polypeptide
DLKPENIMLNHQGHVK

SEQ ID NO: 155 - protein, 16 aa, Artificial Sequence
  Synthetic Polypeptide
DLKPENIMLSSQGHIK

SEQ ID NO: 156 - protein, 12 aa, Artificial Sequence
  Synthetic Polypeptide
VMDPTKILITGK

SEQ ID NO: 157 - protein, 14 aa, Artificial Sequence
  Synthetic Polypeptide
SKLTDNLVALKEIR

SEQ ID NO: 158 - protein, 14 aa, Artificial Sequence
  Synthetic Polypeptide
SKLTENLVALKEIR

SEQ ID NO: 159 - protein, 9 aa, Artificial Sequence
  Synthetic Polypeptide
EYAIKILEK

SEQ ID NO: 160 - protein, 16 aa, Artificial Sequence
  Synthetic Polypeptide
DLKPSNIFFTMDDVVK

SEQ ID NO: 161 - protein, 8 aa, Artificial Sequence
  Synthetic Polypeptide
LVALKVIR

SEQ ID NO: 162 - protein, 16 aa, Artificial Sequence
  Synthetic Polypeptide
DLKPENILLDDNMNIK

SEQ ID NO: 163 - protein, 17 aa, Artificial Sequence
  Synthetic Polypeptide
ATGHEFAVKIMEVTAER

SEQ ID NO: 164 - protein, 14 aa, Artificial Sequence
  Synthetic Polypeptide
SEEPYGQLNPKWTK

SEQ ID NO: 165 - protein, 16 aa, Artificial Sequence
  Synthetic Polypeptide
SGTPMQSAAKAPYLAK

SEQ ID NO: 166 - protein, 14 aa, Artificial Sequence
  Synthetic Polypeptide
VPHTQAVVLNSKDK

SEQ ID NO: 167 - protein, 20 aa, Artificial Sequence
  Synthetic Polypeptide
VIFKCGDDLRQDMLTLQMIR

SEQ ID NO: 168 - protein, 18 aa, Artificial Sequence
  Synthetic Polypeptide
TEDGGKYPVIFKHGDDLR

SEQ ID NO: 169 - protein, 28 aa, Artificial Sequence
  Synthetic Polypeptide
VFGEDSVGVIFKNGDDLRQDMLTLQMLR

SEQ ID NO: 170 - protein, 14 aa, Artificial Sequence
  Synthetic Polypeptide
VNWLAHNVSKDNRQ

SEQ ID NO: 171 - protein, 9 aa, Artificial Sequence
  Synthetic Polypeptide
KKPLWLEFK

SEQ ID NO: 172 - protein, 18 aa, Artificial Sequence
  Synthetic Polypeptide
AKELPTLKDNDFINEGQK

SEQ ID NO: 173 - protein, 18 aa, Artificial Sequence
  Synthetic Polypeptide
AKDLPTFKDNDFLNEGQK

SEQ ID NO: 174 - protein, 28 aa, Artificial Sequence
  Synthetic Polypeptide
TLVIKEVSSEDIADMHSNLSNYHQYIVK

SEQ ID NO: 175 - protein, 32 aa, Artificial Sequence
  Synthetic Polypeptide
EKPLPTFKDLDFLQDIPDGLFLDADMYNALCK

SEQ ID NO: 176 - protein, 19 aa, Artificial Sequence
  Synthetic Polypeptide
GGKSGAAFYATEDDRFILK

SEQ ID NO: 177 - protein, 16 aa, Artificial Sequence
  Synthetic Polypeptide
DLKTSNLLLSHAGILK

SEQ ID NO: 178 - protein, 24 aa, Artificial Sequence
  Synthetic Polypeptide
DLKPENLLIDQQGYIQVTDFGFAK

SEQ ID NO: 179 - protein, 16 aa, Artificial Sequence
  Synthetic Polypeptide
DLKLDNVMLDSEGHIK

SEQ ID NO: 180 - protein, 16 aa, Artificial Sequence
  Synthetic Polypeptide
DLKLDNILLDAEGHCK

SEQ ID NO: 181 - protein, 8 aa, Artificial Sequence
  Synthetic Polypeptide
IYAMKVVK

SEQ ID NO: 182 - protein, 12 aa, Artificial Sequence
  Synthetic Polypeptide
GSFGKVFLAEFK

SEQ ID NO: 183 - protein, 9 aa, Artificial Sequence
  Synthetic Polypeptide
DVAVKVIDK

SEQ ID NO: 184 - protein, 9 aa, Artificial Sequence
  Synthetic Polypeptide
DVAIKVIDK

SEQ ID NO: 185 - protein, 19 aa, Artificial Sequence
  Synthetic Polypeptide
VLLSEFRPSGELFAIKALK

SEQ ID NO: 186 - protein, 16 aa, Artificial Sequence
  Synthetic Polypeptide
DLKLDNLLLDTEGFVK

SEQ ID NO: 187 - protein, 13 aa, Artificial Sequence
  Synthetic Polypeptide
DLKPSNIFLVDTK

SEQ ID NO: 188 - protein, 20 aa, Artificial Sequence
  Synthetic Polypeptide
CFEISDADTKEVFAGKIVPK

SEQ ID NO: 189 - protein, 19 aa, Artificial Sequence
  Synthetic Polypeptide
CNILHADIKPDNILVNESK

SEQ ID NO: 190 - protein, 15 aa, Artificial Sequence
  Synthetic Polypeptide
FLSGLELVKQGAEAR

SEQ ID NO: 191 - protein, 14 aa, Artificial Sequence
  Synthetic Polypeptide
YIEDEDYYKASVTR

SEQ ID NO: 192 - protein, 16 aa, Artificial Sequence
  Synthetic Polypeptide
DLKAENLLLDANLNIK

SEQ ID NO: 193 - protein, 16 aa, Artificial Sequence
  Synthetic Polypeptide
DMKSNNIFLHEGLTVK

SEQ ID NO: 194 - protein, 16 aa, Artificial Sequence
  Synthetic Polypeptide
DLKPSNVLLDPELHVK

SEQ ID NO: 195 - protein, 10 aa, Artificial Sequence
  Synthetic Polypeptide
KLQLELNQER

SEQ ID NO: 196 - protein, 11 aa, Artificial Sequence
  Synthetic Polypeptide
DVKPDNMLLDK

SEQ ID NO: 197 - protein, 31 aa, Artificial Sequence
  Synthetic Polypeptide
DLKPENILLDEEGHIKLTDFGLSKEAIDHEK

SEQ ID NO: 198 - protein, 16 aa, Artificial Sequence
  Synthetic Polypeptide
DLKPENILLDEEGHIK

SEQ ID NO: 199 - protein, 20 aa, Artificial Sequence
  Synthetic Polypeptide
DLKPSNILYVDESGNPECLR

SEQ ID NO: 200 - protein, 31 aa, Artificial Sequence
  Synthetic Polypeptide
DLKPENILLDEEGHIKLTDFGLSKESIDHEK

SEQ ID NO: 201 - protein, 20 aa, Artificial Sequence
  Synthetic Polypeptide
DLKPSNILYVDESGNPESIR

SEQ ID NO: 202 - protein, 24 aa, Artificial Sequence
  Synthetic Polypeptide
DLKPENILLDEEGHIKITDFGLSK

SEQ ID NO: 203 - protein, 16 aa, Artificial Sequence
  Synthetic Polypeptide
DLKPENILLDEIGHIK

SEQ ID NO: 204 - protein, 15 aa, Artificial Sequence
  Synthetic Polypeptide
VLGVIDKVLLVMDTR

SEQ ID NO: 205 - protein, 9 aa, Artificial Sequence
  Synthetic Polypeptide
FYAVKVLQK

SEQ ID NO: 206 - protein, 16 aa, Artificial Sequence
  Synthetic Polypeptide
DLKAGNILFTLDGDIK

SEQ ID NO: 207 - protein, 22 aa, Artificial Sequence
  Synthetic Polypeptide
DTVTIHSVGGTITILPTKTKPK

SEQ ID NO: 208 - protein, 12 aa, Artificial Sequence
  Synthetic Polypeptide
DLKPENVVFFEK

SEQ ID NO: 209 - protein, 25 aa, Artificial Sequence
  Synthetic Polypeptide
VAIKTLKPGTMSPEAFLQEAQVMKK

SEQ ID NO: 210 - protein, 21 aa, Artificial Sequence
  Synthetic Polypeptide
IIHTDIKPENILLSVNEQYIR

SEQ ID NO: 211 - protein, 8 aa, Artificial Sequence
  Synthetic Polypeptide
FVAMKVVK

SEQ ID NO: 212 - protein, 10 aa, Artificial Sequence
  Synthetic Polypeptide
DLKLENIMVK

SEQ ID NO: 213 - protein, 24 aa, Artificial Sequence
  Synthetic Polypeptide
YSVKVLPWLSPEVLQQNLQGYDAK

SEQ ID NO: 214 - protein, 22 aa, Artificial Sequence
  Synthetic Polypeptide
HTPTGTLVTIKITNLENCNEER

SEQ ID NO: 215 - protein, 11 aa, Artificial Sequence
  Synthetic Polypeptide
ISDFGLSKALR

SEQ ID NO: 216 - protein, 17 aa, Artificial Sequence
  Synthetic Polypeptide
DLKPPNLLLVAGGTVLK

SEQ ID NO: 217 - protein, 16 aa, Artificial Sequence
  Synthetic Polypeptide
DIKAGNILLTEPGQVK

SEQ ID NO: 218 - protein, 16 aa, Artificial Sequence
  Synthetic Polypeptide
DVKAGNILLSEPGLVK

SEQ ID NO: 219 - protein, 24 aa, Artificial Sequence
  Synthetic Polypeptide
TGDLFAIKVFNNISFLRPVDVQMR

SEQ ID NO: 220 - protein, 18 aa, Artificial Sequence
  Synthetic Polypeptide
YVLDDQYTSSSGAKFPVK

SEQ ID NO: 221 - protein, 31 aa, Artificial Sequence
  Synthetic Polypeptide
YLNEIKPPIIHYDLKPGNILLVDGTACGEIK

SEQ ID NO: 222 - protein, 31 aa, Artificial Sequence
  Synthetic Polypeptide
YLNEIKPPIIHYDLKPGNILLVNGTACGEIK

SEQ ID NO: 223 - protein, 18 aa, Artificial Sequence
  Synthetic Polypeptide
IGDFGLAKAVPEGHEYYR

SEQ ID NO: 224 - protein, 15 aa, Artificial Sequence
  Synthetic Polypeptide
DLKPQNILLSNPAGR

SEQ ID NO: 225 - protein, 23 aa, Artificial Sequence
  Synthetic Polypeptide
NISHLDLKPQNILLSSLEKPHLK

SEQ ID NO: 226 - protein, 28 aa, Artificial Sequence
  Synthetic Polypeptide
MLDVLEYIHENEYVHGDIKAANLLLGYK

SEQ ID NO: 227 - protein, 21 aa, Artificial Sequence
  Synthetic Polypeptide
YIHSMSLVHMDIKPSNIFISR

SEQ ID NO: 228 - protein, 8 aa, Artificial Sequence
  Synthetic Polypeptide
GSFKTVYK

SEQ ID NO: 229 - protein, 17 aa, Artificial Sequence
  Synthetic Polypeptide
DLKCDNIFITGPTGSVK

SEQ ID NO: 230 - protein, 12 aa, Artificial Sequence
  Synthetic Polypeptide
DVKPDNILLDER

SEQ ID NO: 231 - protein, 37 aa, Artificial Sequence
  Synthetic Polypeptide
EVVAIKIIDLEEAEDEIEDIQQEITVLSQCDSPYITR

SEQ ID NO: 232 - protein, 12 aa, Artificial Sequence
  Synthetic Polypeptide
WISQDKEVAVKK

SEQ ID NO: 233 - protein, 29 aa, Artificial Sequence
  Synthetic Polypeptide
TGQLAAIKVMDVTEDEEEEIKLEINMLKK

SEQ ID NO: 234 - protein, 16 aa, Artificial Sequence
  Synthetic Polypeptide
DIKGQNVLLTENAEVK

SEQ ID NO: 235 - protein, 29 aa, Artificial Sequence
  Synthetic Polypeptide
TGQLAAIKVMDVTGDEEEEIKQEINMLKK